European Patent Specification EP 4 149 548 B1, published April 29, 2026. Title: ANTI-HEMOJUVELIN (HJV) ANTIBODIES FOR TREATING MYELOFIBROSIS. Applicant: Disc Medicine, Inc AbbVie Deutschland GmbH & Co. KG AbbVie Inc. Application Not Yet Assigned. The sequence listing filed with the application follows.

SEQUENCE LISTING (129 sequences)

SEQ ID NO: 1 - protein, 5 aa, Artificial Sequence
  Synthethic Polypeptide
NYGMN

SEQ ID NO: 2 - protein, 17 aa, Artificial Sequence
  Synthethic Polypeptide
MIYYDSSEKHYADSVKG

SEQ ID NO: 3 - protein, 6 aa, Artificial Sequence
  Synthethic Polypeptide
GTTPDY

SEQ ID NO: 4 - protein, 16 aa, Artificial Sequence
  Synthethic Polypeptide
RSSQSLETSDGDTFLE

SEQ ID NO: 5 - protein, 7 aa, Artificial Sequence
  Synthethic Polypeptide
EVSTRFS

SEQ ID NO: 6 - protein, 9 aa, Artificial Sequence
  Synthethic Polypeptide
FQVTHDPMT

SEQ ID NO: 7 - protein, 115 aa, Artificial Sequence
  Synthethic Polypeptide
EVQLVESGGGLVQPGGSLRLSCAASGFTFSNYGMNWIRQAPGKGLEWIGMIYYDSSEKHYADSVKGRFTISRDNSKNTLYLQMNSLRAEDTAVYYCAKGTTPDYWGQGTMVTVSS

SEQ ID NO: 8 - protein, 112 aa, Artificial Sequence
  Synthethic Polypeptide
DVVLTQSPLSLPVTLGQPASISCRSSQSLETSDGDTFLEWFQQRPGQSPRLLIYEVSTRFSGVPDRFSGSGSGTDFTLKISRVEAEDVGVYYCFQVTHDPMTFGQGTKLEIK

SEQ ID NO: 9 - protein, 5 aa, Artificial Sequence
  Synthethic Polypeptide
YYGMN

SEQ ID NO: 10 - protein, 17 aa, Artificial Sequence
  Synthethic Polypeptide
MIYYDSSDKHYADSVKG

SEQ ID NO: 11 - protein, 6 aa, Artificial Sequence
  Synthethic Polypeptide
GTTPDV

SEQ ID NO: 12 - protein, 6 aa, Artificial Sequence
  Synthethic Polypeptide
GTTPDK

SEQ ID NO: 13 - protein, 6 aa, Artificial Sequence
  Synthethic Polypeptide
GSTPDY

SEQ ID NO: 14 - protein, 16 aa, Artificial Sequence
  Synthethic Polypeptide
RSSQSLESSDGDTFLE

SEQ ID NO: 15 - protein, 16 aa, Artificial Sequence
  Synthethic Polypeptide
RSSQSLEESDGYTFLE

SEQ ID NO: 16 - protein, 16 aa, Artificial Sequence
  Synthethic Polypeptide
RSSQSLEDSDGGTFLE

SEQ ID NO: 17 - protein, 16 aa, Artificial Sequence
  Synthethic Polypeptide
RSSQSLEESDGYTFLH

SEQ ID NO: 18 - protein, 7 aa, Artificial Sequence
  Synthethic Polypeptide
EVSNRFS

SEQ ID NO: 19 - protein, 7 aa, Artificial Sequence
  Synthethic Polypeptide
DVSTRFS

SEQ ID NO: 20 - protein, 7 aa, Artificial Sequence
  Synthethic Polypeptide
DVSERFS

SEQ ID NO: 21 - protein, 7 aa, Artificial Sequence
  Synthethic Polypeptide
DVSSRFS

SEQ ID NO: 22 - protein, 7 aa, Artificial Sequence
  Synthethic Polypeptide
AVSHRFS

SEQ ID NO: 23 - protein, 7 aa, Artificial Sequence
  Synthethic Polypeptide
EVSHRFS

SEQ ID NO: 24 - protein, 9 aa, Artificial Sequence
  Synthethic Polypeptide
MQVTHDPLT

SEQ ID NO: 25 - protein, 9 aa, Artificial Sequence
  Synthethic Polypeptide
FQVTHDPVT

SEQ ID NO: 26 - protein, 9 aa, Artificial Sequence
  Synthethic Polypeptide
FQATYDPLT

SEQ ID NO: 27 - protein, 9 aa, Artificial Sequence
  Synthethic Polypeptide
FQATHDPLT

SEQ ID NO: 28 - protein, 9 aa, Artificial Sequence
  Synthethic Polypeptide
FQATHDPVT

SEQ ID NO: 29 - protein, 9 aa, Artificial Sequence
  Synthethic Polypeptide
FQATHDPLS

SEQ ID NO: 30 - protein, 112 aa, Artificial Sequence
  Synthethic Polypeptide
DVVLTQSPLSLPVTLGQPASISCRSSQSLETSDGDTFLEWFQQRPGQSPRLLIYEVSSRFSGVPDRFSGSGSGTDFTLKISRVEAEDVGVYYCMQVTHDPLTFGQGTKLEIK

SEQ ID NO: 31 - protein, 112 aa, Artificial Sequence
  Synthethic Polypeptide
DVVLTQSPLSLPVTLGQPASISCRSSQSLETSDGDTFLEWFQQRPGQSPRLLIYEVSNRFSGVPDRFSGSGSGTDFTLKISRVEAEDVGVYYCFQVTHDPVTFGQGTKLEIK

SEQ ID NO: 32 - protein, 112 aa, Artificial Sequence
  Synthethic Polypeptide
DVVLTQSPLSLPVTLGQPASISCRSSQSLESSDGDTFLEWFQQRPGQSPRLLIYDVSTRFSGVPDRFSGSGSGTDFTLKISRVEAEDVGVYYCFQVTHDPVTFGQGTKLEIK

SEQ ID NO: 33 - protein, 112 aa, Artificial Sequence
  Synthethic Polypeptide
DVVLTQSPLSLPVTLGQPASISCRSSQSLEESDGYTFLEWFQQRPGQSPRLLIYDVSERFSGVPDRFSGSGSGTDFTLKISRVEAEDVGVYYCFQATYDPLTFGQGTKLEIK

SEQ ID NO: 34 - protein, 115 aa, Artificial Sequence
  Synthethic Polypeptide
EVQLVESGGGLVQPGGSLRLSCAASGFTFSYYGMNWIRQAPGKGLEWIGMIYYDSSEKHYADSVKGRFTISRDNSKNTLYLQMNSLRAEDTAVYYCAKGTTPDYWGQGTMVTVSS

SEQ ID NO: 35 - protein, 112 aa, Artificial Sequence
  Synthethic Polypeptide
DVVLTQSPLSLPVTLGQPASISCRSSQSLEDSDGGTFLEWFQQRPGQSPRLLIYDVSSRFSGVPDRFSGSGSGTDFTLKISRVEAEDVGVYYCFQATHDPLTFGQGTKLEIK

SEQ ID NO: 36 - protein, 115 aa, Artificial Sequence
  Synthethic Polypeptide
EVQLVESGGGLVQPGGSLRLSCAASGFTFSNYGMNWIRQAPGKGLEWIGMIYYDSSDKHYADSVKGRFTISRDNSKNTLYLQMNSLRAEDTAVYYCAKGTTPDVWGQGTMVTVSS

SEQ ID NO: 37 - protein, 112 aa, Artificial Sequence
  Synthethic Polypeptide
DVVLTQSPLSLPVTLGQPASISCRSSQSLEESDGYTFLHWFQQRPGQSPRLLIYEVSNRFSGVPDRFSGSGSGTDFTLKISRVEAEDVGVYYCFQATHDPVTFGQGTKLEIK

SEQ ID NO: 38 - protein, 115 aa, Artificial Sequence
  Synthethic Polypeptide
EVQLVESGGGLVQPGGSLRLSCAASGFTFSNYGMNWVRQAPGKGLEWIGMIYYDSSEKHYADSVKGRFTISRDNSKNTLYLQMNSLRAEDTAVYYCAKGTTPDYWGQGTMVTVSS

SEQ ID NO: 39 - protein, 112 aa, Artificial Sequence
  Synthethic Polypeptide
DVVLTQSPLSLPVTLGQPASISCRSSQSLEESDGYTFLHWFQQRPGQSPRLLIYEVSTRFSGVPDRFSGSGSGTDFTLKISRVEAEDVGVYYCFQATHDPLTFGQGTKLEIK

SEQ ID NO: 40 - DNA, 1338 bp, Artificial Sequence
  Synthethic Polynucleotide
gaagtacagttggtagaaagcggcggaggacttgtgcagccaggtggatctctcagactttcatgtgccgcaagcggttttacttttagtaactatggaatgaactgggttagacaagcgcccggaaaaggattggaatggataggaatgatatactacgacagctccgagaaacattatgccgactcagttaaaggaagatttacaatatcaagagacaatagcaaaaacacactttatcttcaaatgaattcactgcgagccgaggatacagcagtctattattgcgcaaaaggctcgacccccgattactggggtcaaggaacaatggtaaccgtgtcaagcgcgtcgaccaagggcccatcggtcttccccctggcaccctcctccaagagcacctctgggggcacagcggccctgggctgcctggtcaaggactacttccccgaaccggtgacggtgtcgtggaactcaggcgccctgaccagcggcgtgcacaccttcccggctgtcctacagtcctcaggactctactccctcagcagcgtggtgaccgtgccctccagcagcttgggcacccagacctacatctgcaacgtgaatcacaagcccagcaacaccaaggtggacaagaaagttgagcccaaatcttgtgacaaaactcacacatgcccaccgtgcccagcacctgaagccgcggggggaccgtcagtcttcctcttccccccaaaacccaaggacaccctcatgatctcccggacccctgaggtcacatgcgtggtggtggacgtgagccacgaagaccctgaggtcaagttcaactggtacgtggacggcgtggaggtgcataatgccaagacaaagccgcgggaggagcagtacaacagcacgtaccgtgtggtcagcgtcctcaccgtcctgcaccaggactggctgaatggcaaggagtacaagtgcaaggtctccaacaaagccctcccagcccccatcgagaaaaccatctccaaagccaaagggcagccccgagaaccacaggtgtacaccctgcccccatcccgcgaggagatgaccaagaaccaggtcagcctgacctgcctggtcaaaggcttctatcccagcgacatcgccgtggagtgggagagcaatgggcagccggagaacaactacaagaccacgcctcccgtgctggactccgacggctccttcttcctctacagcaagctcaccgtggacaagagcaggtggcagcaggggaacgtcttctcatgctccgtgatgcatgaggctctgcacaaccactacacgcagaagagcctctccctgtctccgggtaaatga

SEQ ID NO: 41 - protein, 112 aa, Artificial Sequence
  Synthethic Polypeptide
DVVLTQSPLSLPVTLGQPASISCRSSQSLADSDGDTFLHWFQQRPGQSPRLLIYAVSHRFSGVPDRFSGSGSGTDFTLKISRVEAEDVGVYYCFQATHDPVTFGQGTKLEIK

SEQ ID NO: 42 - protein, 115 aa, Artificial Sequence
  Synthethic Polypeptide
EVQLVESGGGLVQPGGSLRLSCAASGFTFSNYGMNWVRQAPGKGLEWIGMIYYDSSEKHYADSVKGRFTISRDNSKNTLYLQMNSLRAEDTAVYYCAKGTTPDKWGQGTMVTVSS

SEQ ID NO: 43 - protein, 112 aa, Artificial Sequence
  Synthethic Polypeptide
DVVLTQSPLSLPVTLGQPASISCRSSQSLEESDGYTFLEWFQQRPGQSPRLLIYEVSHRFSGVPDRFSGSGSGTDFTLKISRVEAEDVGVYYCFQATHDPLTFGQGTKLEIK

SEQ ID NO: 44 - protein, 115 aa, Artificial Sequence
  Synthethic Polypeptide
EVQLVESGGGLVQPGGSLRLSCAASGFTFSNYGMNWVRQAPGKGLEWIGMIYYDSSEKHYADSVKGRFTISRDNSKNTLYLQMNSLRAEDTAVYYCAKGSTPDYWGQGTMVTVSS

SEQ ID NO: 45 - protein, 112 aa, Artificial Sequence
  Synthethic Polypeptide
DVVLTQSPLSLPVTLGQPASISCRSSQSLEDSDGGTFLEWFQQRPGQSPRLLIYDVSSRFSGVPDRFSGSGSGTDFTLKISRVEAEDVGVYYCFQATHDPLSFGQGTKLEIK

SEQ ID NO: 46 - protein, 330 aa, Artificial Sequence
  Synthethic Polypeptide
ASTKGPSVFPLAPSSKSTSGGTAALGCLVKDYFPEPVTVSWNSGALTSGVHTFPAVLQSSGLYSLSSVVTVPSSSLGTQTYICNVNHKPSNTKVDKKVEPKSCDKTHTCPPCPAPEAAGGPSVFLFPPKPKDTLMISRTPEVTCVVVDVSHEDPEVKFNWYVDGVEVHNAKTKPREEQYNSTYRVVSVLTVLHQDWLNGKEYKCKVSNKALPAPIEKTISKAKGQPREPQVYTLPPSREEMTKNQVSLTCLVKGFYPSDIAVEWESNGQPENNYKTTPPVLDSDGSFFLYSKLTVDKSRWQQGNVFSCSVMHEALHNHYTQKSLSLSPGK

SEQ ID NO: 47 - protein, 107 aa, Homo sapiens [sequence omitted]

SEQ ID NO: 48 - protein, 330 aa, Artificial Sequence
  Synthetic Polypeptide
ASTKGPSVFPLAPSSKSTSGGTAALGCLVKDYFPEPVTVSWNSGALTSGVHTFPAVLQSSGLYSLSSVVTVPSSSLGTQTYICNVNHKPSNTKVDKKVEPKSCDKTHTCPPCPAPEAAGGPSVFLFPPKPKDQLMISRTPEVTCVVVDVSHEDPEVKFNWYVDGVEVHNAKTKPREEQYNSTYRVVSVLTVLHQDWLNGKEYKCKVSNKALPAPIEKTISKAKGQPREPQVYTLPPSREEMTKNQVSLTCLVKGFYPSDIAVEWESNGQPENNYKTTPPVLDSDGSFFLYSKLTVDKSRWQQGNVFSCSVLHEALHNHYTQKSLSLSPGK

SEQ ID NO: 49 - protein, 7 aa, Artificial Sequence
  Synthethic Polypeptide
EVSSRFS

SEQ ID NO: 50 - protein, 16 aa, Artificial Sequence
  Synthethic Polypeptide
RSSQSLADSDGDTFLH

SEQ ID NO: 51 - protein, 445 aa, Artificial Sequence
  Synthethic Polypeptide
EVQLVESGGGLVQPGGSLRLSCAASGFTFSNYGMNWIRQAPGKGLEWIGMIYYDSSEKHYADSVKGRFTISRDNSKNTLYLQMNSLRAEDTAVYYCAKGTTPDYWGQGTMVTVSSASTKGPSVFPLAPSSKSTSGGTAALGCLVKDYFPEPVTVSWNSGALTSGVHTFPAVLQSSGLYSLSSVVTVPSSSLGTQTYICNVNHKPSNTKVDKKVEPKSCDKTHTCPPCPAPEAAGGPSVFLFPPKPKDTLMISRTPEVTCVVVDVSHEDPEVKFNWYVDGVEVHNAKTKPREEQYNSTYRVVSVLTVLHQDWLNGKEYKCKVSNKALPAPIEKTISKAKGQPREPQVYTLPPSREEMTKNQVSLTCLVKGFYPSDIAVEWESNGQPENNYKTTPPVLDSDGSFFLYSKLTVDKSRWQQGNVFSCSVMHEALHNHYTQKSLSLSPGK

SEQ ID NO: 52 - protein, 219 aa, Artificial Sequence
  Synthethic Polypeptide
DVVLTQSPLSLPVTLGQPASISCRSSQSLETSDGDTFLEWFQQRPGQSPRLLIYEVSTRFSGVPDRFSGSGSGTDFTLKISRVEAEDVGVYYCFQVTHDPMTFGQGTKLEIKRTVAAPSVFIFPPSDEQLKSGTASVVCLLNNFYPREAKVQWKVDNALQSGNSQESVTEQDSKDSTYSLSSTLTLSKADYEKHKVYACEVTHQGLSSPVTKSFNRGEC

SEQ ID NO: 53 - protein, 219 aa, Artificial Sequence
  Synthethic Polypeptide
DVVLTQSPLSLPVTLGQPASISCRSSQSLETSDGDTFLEWFQQRPGQSPRLLIYEVSSRFSGVPDRFSGSGSGTDFTLKISRVEAEDVGVYYCMQVTHDPLTFGQGTKLEIKRTVAAPSVFIFPPSDEQLKSGTASVVCLLNNFYPREAKVQWKVDNALQSGNSQESVTEQDSKDSTYSLSSTLTLSKADYEKHKVYACEVTHQGLSSPVTKSFNRGEC

SEQ ID NO: 54 - protein, 219 aa, Artificial Sequence
  Synthethic Polypeptide
DVVLTQSPLSLPVTLGQPASISCRSSQSLETSDGDTFLEWFQQRPGQSPRLLIYEVSNRFSGVPDRFSGSGSGTDFTLKISRVEAEDVGVYYCFQVTHDPVTFGQGTKLEIKRTVAAPSVFIFPPSDEQLKSGTASVVCLLNNFYPREAKVQWKVDNALQSGNSQESVTEQDSKDSTYSLSSTLTLSKADYEKHKVYACEVTHQGLSSPVTKSFNRGEC

SEQ ID NO: 55 - protein, 219 aa, Artificial Sequence
  Synthethic Polypeptide
DVVLTQSPLSLPVTLGQPASISCRSSQSLESSDGDTFLEWFQQRPGQSPRLLIYDVSTRFSGVPDRFSGSGSGTDFTLKISRVEAEDVGVYYCFQVTHDPVTFGQGTKLEIKRTVAAPSVFIFPPSDEQLKSGTASVVCLLNNFYPREAKVQWKVDNALQSGNSQESVTEQDSKDSTYSLSSTLTLSKADYEKHKVYACEVTHQGLSSPVTKSFNRGEC

SEQ ID NO: 56 - protein, 219 aa, Artificial Sequence
  Synthethic Polypeptide
DVVLTQSPLSLPVTLGQPASISCRSSQSLEESDGYTFLEWFQQRPGQSPRLLIYDVSERFSGVPDRFSGSGSGTDFTLKISRVEAEDVGVYYCFQATYDPLTFGQGTKLEIKRTVAAPSVFIFPPSDEQLKSGTASVVCLLNNFYPREAKVQWKVDNALQSGNSQESVTEQDSKDSTYSLSSTLTLSKADYEKHKVYACEVTHQGLSSPVTKSFNRGEC

SEQ ID NO: 57 - protein, 445 aa, Artificial Sequence
  Synthethic Polypeptide
EVQLVESGGGLVQPGGSLRLSCAASGFTFSYYGMNWIRQAPGKGLEWIGMIYYDSSEKHYADSVKGRFTISRDNSKNTLYLQMNSLRAEDTAVYYCAKGTTPDYWGQGTMVTVSSASTKGPSVFPLAPSSKSTSGGTAALGCLVKDYFPEPVTVSWNSGALTSGVHTFPAVLQSSGLYSLSSVVTVPSSSLGTQTYICNVNHKPSNTKVDKKVEPKSCDKTHTCPPCPAPEAAGGPSVFLFPPKPKDTLMISRTPEVTCVVVDVSHEDPEVKFNWYVDGVEVHNAKTKPREEQYNSTYRVVSVLTVLHQDWLNGKEYKCKVSNKALPAPIEKTISKAKGQPREPQVYTLPPSREEMTKNQVSLTCLVKGFYPSDIAVEWESNGQPENNYKTTPPVLDSDGSFFLYSKLTVDKSRWQQGNVFSCSVMHEALHNHYTQKSLSLSPGK

SEQ ID NO: 58 - protein, 219 aa, Artificial Sequence
  Synthethic Polypeptide
DVVLTQSPLSLPVTLGQPASISCRSSQSLEDSDGGTFLEWFQQRPGQSPRLLIYDVSSRFSGVPDRFSGSGSGTDFTLKISRVEAEDVGVYYCFQATHDPLTFGQGTKLEIKRTVAAPSVFIFPPSDEQLKSGTASVVCLLNNFYPREAKVQWKVDNALQSGNSQESVTEQDSKDSTYSLSSTLTLSKADYEKHKVYACEVTHQGLSSPVTKSFNRGEC

SEQ ID NO: 59 - protein, 445 aa, Artificial Sequence
  Synthethic Polypeptide
EVQLVESGGGLVQPGGSLRLSCAASGFTFSNYGMNWIRQAPGKGLEWIGMIYYDSSDKHYADSVKGRFTISRDNSKNTLYLQMNSLRAEDTAVYYCAKGTTPDVWGQGTMVTVSSASTKGPSVFPLAPSSKSTSGGTAALGCLVKDYFPEPVTVSWNSGALTSGVHTFPAVLQSSGLYSLSSVVTVPSSSLGTQTYICNVNHKPSNTKVDKKVEPKSCDKTHTCPPCPAPEAAGGPSVFLFPPKPKDTLMISRTPEVTCVVVDVSHEDPEVKFNWYVDGVEVHNAKTKPREEQYNSTYRVVSVLTVLHQDWLNGKEYKCKVSNKALPAPIEKTISKAKGQPREPQVYTLPPSREEMTKNQVSLTCLVKGFYPSDIAVEWESNGQPENNYKTTPPVLDSDGSFFLYSKLTVDKSRWQQGNVFSCSVMHEALHNHYTQKSLSLSPGK

SEQ ID NO: 60 - protein, 219 aa, Artificial Sequence
  Synthethic Polypeptide
DVVLTQSPLSLPVTLGQPASISCRSSQSLEESDGYTFLHWFQQRPGQSPRLLIYEVSNRFSGVPDRFSGSGSGTDFTLKISRVEAEDVGVYYCFQATHDPVTFGQGTKLEIKRTVAAPSVFIFPPSDEQLKSGTASVVCLLNNFYPREAKVQWKVDNALQSGNSQESVTEQDSKDSTYSLSSTLTLSKADYEKHKVYACEVTHQGLSSPVTKSFNRGEC

SEQ ID NO: 61 - protein, 445 aa, Artificial Sequence
  Synthethic Polypeptide
EVQLVESGGGLVQPGGSLRLSCAASGFTFSNYGMNWVRQAPGKGLEWIGMIYYDSSEKHYADSVKGRFTISRDNSKNTLYLQMNSLRAEDTAVYYCAKGTTPDYWGQGTMVTVSSASTKGPSVFPLAPSSKSTSGGTAALGCLVKDYFPEPVTVSWNSGALTSGVHTFPAVLQSSGLYSLSSVVTVPSSSLGTQTYICNVNHKPSNTKVDKKVEPKSCDKTHTCPPCPAPEAAGGPSVFLFPPKPKDTLMISRTPEVTCVVVDVSHEDPEVKFNWYVDGVEVHNAKTKPREEQYNSTYRVVSVLTVLHQDWLNGKEYKCKVSNKALPAPIEKTISKAKGQPREPQVYTLPPSREEMTKNQVSLTCLVKGFYPSDIAVEWESNGQPENNYKTTPPVLDSDGSFFLYSKLTVDKSRWQQGNVFSCSVMHEALHNHYTQKSLSLSPGK

SEQ ID NO: 62 - protein, 219 aa, Artificial Sequence
  Synthethic Polypeptide
DVVLTQSPLSLPVTLGQPASISCRSSQSLEESDGYTFLHWFQQRPGQSPRLLIYEVSTRFSGVPDRFSGSGSGTDFTLKISRVEAEDVGVYYCFQATHDPLTFGQGTKLEIKRTVAAPSVFIFPPSDEQLKSGTASVVCLLNNFYPREAKVQWKVDNALQSGNSQESVTEQDSKDSTYSLSSTLTLSKADYEKHKVYACEVTHQGLSSPVTKSFNRGEC

SEQ ID NO: 63 - protein, 445 aa, Artificial Sequence
  Synthethic Polypeptide
EVQLVESGGGLVQPGGSLRLSCAASGFTFSNYGMNWVRQAPGKGLEWIGMIYYDSSEKHYADSVKGRFTISRDNSKNTLYLQMNSLRAEDTAVYYCAKGTTPDYWGQGTMVTVSSASTKGPSVFPLAPSSKSTSGGTAALGCLVKDYFPEPVTVSWNSGALTSGVHTFPAVLQSSGLYSLSSVVTVPSSSLGTQTYICNVNHKPSNTKVDKKVEPKSCDKTHTCPPCPAPEAAGGPSVFLFPPKPKDQLMISRTPEVTCVVVDVSHEDPEVKFNWYVDGVEVHNAKTKPREEQYNSTYRVVSVLTVLHQDWLNGKEYKCKVSNKALPAPIEKTISKAKGQPREPQVYTLPPSREEMTKNQVSLTCLVKGFYPSDIAVEWESNGQPENNYKTTPPVLDSDGSFFLYSKLTVDKSRWQQGNVFSCSVLHEALHNHYTQKSLSLSPGK

SEQ ID NO: 64 - DNA, 660 bp, Artificial Sequence
  Synthethic Polynucleotide
gacgtagtactgacccaaagccccctttctctcccagtaaccctcggacaaccagcctcaatttcatgcagatcatcacaatcacttgaggacagcgacggaggcacttttcttgagtggttccaacaaagacccggacaaagcccacgcctgcttatttacgacgtatcaagcagattctcaggagttccagacagattttcaggcagcggatccggcacagacttcacccttaaaattagcagagtagaagcagaagatgtaggagtgtattattgtttccaagccacccacgaccccctcagcttcggacaaggaactaagctcgaaatcaaaagaacggtggctgcaccatctgtcttcatcttcccgccatctgatgagcagttgaaatctggaactgcctctgttgtgtgcctgctgaataacttctatcccagagaggccaaagtacagtggaaggtggataacgccctccaatcgggtaactcccaggagagtgtcacagagcaggacagcaaggacagcacctacagcctcagcagcaccctgacgctgagcaaagcagactacgagaaacacaaagtctacgcctgcgaagtcacccatcagggcctgagctcgcccgtcacaaagagcttcaacaggggagagtgttga

SEQ ID NO: 65 - protein, 219 aa, Artificial Sequence
  Synthethic Polypeptide
DVVLTQSPLSLPVTLGQPASISCRSSQSLADSDGDTFLHWFQQRPGQSPRLLIYAVSHRFSGVPDRFSGSGSGTDFTLKISRVEAEDVGVYYCFQATHDPVTFGQGTKLEIKRTVAAPSVFIFPPSDEQLKSGTASVVCLLNNFYPREAKVQWKVDNALQSGNSQESVTEQDSKDSTYSLSSTLTLSKADYEKHKVYACEVTHQGLSSPVTKSFNRGEC

SEQ ID NO: 66 - protein, 445 aa, Artificial Sequence
  Synthethic Polypeptide
EVQLVESGGGLVQPGGSLRLSCAASGFTFSNYGMNWVRQAPGKGLEWIGMIYYDSSEKHYADSVKGRFTISRDNSKNTLYLQMNSLRAEDTAVYYCAKGTTPDKWGQGTMVTVSSASTKGPSVFPLAPSSKSTSGGTAALGCLVKDYFPEPVTVSWNSGALTSGVHTFPAVLQSSGLYSLSSVVTVPSSSLGTQTYICNVNHKPSNTKVDKKVEPKSCDKTHTCPPCPAPEAAGGPSVFLFPPKPKDTLMISRTPEVTCVVVDVSHEDPEVKFNWYVDGVEVHNAKTKPREEQYNSTYRVVSVLTVLHQDWLNGKEYKCKVSNKALPAPIEKTISKAKGQPREPQVYTLPPSREEMTKNQVSLTCLVKGFYPSDIAVEWESNGQPENNYKTTPPVLDSDGSFFLYSKLTVDKSRWQQGNVFSCSVMHEALHNHYTQKSLSLSPGK

SEQ ID NO: 67 - protein, 219 aa, Artificial Sequence
  Synthethic Polypeptide
DVVLTQSPLSLPVTLGQPASISCRSSQSLEESDGYTFLEWFQQRPGQSPRLLIYEVSHRFSGVPDRFSGSGSGTDFTLKISRVEAEDVGVYYCFQATHDPLTFGQGTKLEIKRTVAAPSVFIFPPSDEQLKSGTASVVCLLNNFYPREAKVQWKVDNALQSGNSQESVTEQDSKDSTYSLSSTLTLSKADYEKHKVYACEVTHQGLSSPVTKSFNRGEC

SEQ ID NO: 68 - protein, 445 aa, Artificial Sequence
  Synthethic Polypeptide
EVQLVESGGGLVQPGGSLRLSCAASGFTFSNYGMNWVRQAPGKGLEWIGMIYYDSSEKHYADSVKGRFTISRDNSKNTLYLQMNSLRAEDTAVYYCAKGSTPDYWGQGTMVTVSSASTKGPSVFPLAPSSKSTSGGTAALGCLVKDYFPEPVTVSWNSGALTSGVHTFPAVLQSSGLYSLSSVVTVPSSSLGTQTYICNVNHKPSNTKVDKKVEPKSCDKTHTCPPCPAPEAAGGPSVFLFPPKPKDTLMISRTPEVTCVVVDVSHEDPEVKFNWYVDGVEVHNAKTKPREEQYNSTYRVVSVLTVLHQDWLNGKEYKCKVSNKALPAPIEKTISKAKGQPREPQVYTLPPSREEMTKNQVSLTCLVKGFYPSDIAVEWESNGQPENNYKTTPPVLDSDGSFFLYSKLTVDKSRWQQGNVFSCSVMHEALHNHYTQKSLSLSPGK

SEQ ID NO: 69 - protein, 219 aa, Artificial Sequence
  Synthethic Polypeptide
DVVLTQSPLSLPVTLGQPASISCRSSQSLEDSDGGTFLEWFQQRPGQSPRLLIYDVSSRFSGVPDRFSGSGSGTDFTLKISRVEAEDVGVYYCFQATHDPLSFGQGTKLEIKRTVAAPSVFIFPPSDEQLKSGTASVVCLLNNFYPREAKVQWKVDNALQSGNSQESVTEQDSKDSTYSLSSTLTLSKADYEKHKVYACEVTHQGLSSPVTKSFNRGEC

SEQ ID NO: 70 - DNA, 345 bp, Artificial Sequence
  Synthethic Polynucleotide
gaagtacagttggtagaaagcggcggaggacttgtgcagccaggtggatctctcagactttcatgtgccgcaagcggttttacttttagtaactatggaatgaattggattagacaagcgcccggaaaaggattggaatggataggaatgatatactacgatagctcagaaaaacattatgccgactcagttaaaggaagatttacaatatcaagagacaatagcaaaaacacactttatcttcaaatgaattcactgcgagccgaggatacagcagtctattattgcgcaaaaggaacaacaccagattattggggtcaaggaacaatggtaaccgtgtcaagc

SEQ ID NO: 71 - DNA, 1338 bp, Artificial Sequence
  Synthethic Polynucleotide
gaagtacagttggtagaaagcggcggaggacttgtgcagccaggtggatctctcagactttcatgtgccgcaagcggttttacttttagtaactatggaatgaattggattagacaagcgcccggaaaaggattggaatggataggaatgatatactacgatagctcagaaaaacattatgccgactcagttaaaggaagatttacaatatcaagagacaatagcaaaaacacactttatcttcaaatgaattcactgcgagccgaggatacagcagtctattattgcgcaaaaggaacaacaccagattattggggtcaaggaacaatggtaaccgtgtcaagcgcgtcgaccaagggcccatcggtcttccccctggcaccctcctccaagagcacctctgggggcacagcggccctgggctgcctggtcaaggactacttccccgaaccggtgacggtgtcgtggaactcaggcgccctgaccagcggcgtgcacaccttcccggctgtcctacagtcctcaggactctactccctcagcagcgtggtgaccgtgccctccagcagcttgggcacccagacctacatctgcaacgtgaatcacaagcccagcaacaccaaggtggacaagaaagttgagcccaaatcttgtgacaaaactcacacatgcccaccgtgcccagcacctgaagccgcggggggaccgtcagtcttcctcttccccccaaaacccaaggacaccctcatgatctcccggacccctgaggtcacatgcgtggtggtggacgtgagccacgaagaccctgaggtcaagttcaactggtacgtggacggcgtggaggtgcataatgccaagacaaagccgcgggaggagcagtacaacagcacgtaccgtgtggtcagcgtcctcaccgtcctgcaccaggactggctgaatggcaaggagtacaagtgcaaggtctccaacaaagccctcccagcccccatcgagaaaaccatctccaaagccaaagggcagccccgagaaccacaggtgtacaccctgcccccatcccgcgaggagatgaccaagaaccaggtcagcctgacctgcctggtcaaaggcttctatcccagcgacatcgccgtggagtgggagagcaatgggcagccggagaacaactacaagaccacgcctcccgtgctggactccgacggctccttcttcctctacagcaagctcaccgtggacaagagcaggtggcagcaggggaacgtcttctcatgctccgtgatgcatgaggctctgcacaaccactacacgcagaagagcctctccctgtctccgggtaaatga

SEQ ID NO: 72 - DNA, 336 bp, Artificial Sequence
  Synthethic Polynucleotide
gacgtagtactgacccaaagccccctttctctcccagtaaccctcggacaaccagcctcaatttcatgcagatcatcacaatcacttgagacgagcgacggagacacttttcttgagtggttccaacaaagacccggacaaagcccacgcctgcttatttacgaggtatcaacgagattctcaggagttccagacagattttcaggcagcggatccggcacagacttcacccttaaaattagcagagtagaagcagaagatgtaggagtgtattattgttttcaagtcacccacgaccccatgacgttcggacaaggaactaagctcgaaatcaaa

SEQ ID NO: 73 - DNA, 660 bp, Artificial Sequence
  Synthethic Polynucleotide
gacgtagtactgacccaaagccccctttctctcccagtaaccctcggacaaccagcctcaatttcatgcagatcatcacaatcacttgagacgagcgacggagacacttttcttgagtggttccaacaaagacccggacaaagcccacgcctgcttatttacgaggtatcaacgagattctcaggagttccagacagattttcaggcagcggatccggcacagacttcacccttaaaattagcagagtagaagcagaagatgtaggagtgtattattgttttcaagtcacccacgaccccatgacgttcggacaaggaactaagctcgaaatcaaaagaacggtggctgcaccatctgtcttcatcttcccgccatctgatgagcagttgaaatctggaactgcctctgttgtgtgcctgctgaataacttctatcccagagaggccaaagtacagtggaaggtggataacgccctccaatcgggtaactcccaggagagtgtcacagagcaggacagcaaggacagcacctacagcctcagcagcaccctgacgctgagcaaagcagactacgagaaacacaaagtctacgcctgcgaagtcacccatcagggcctgagctcgcccgtcacaaagagcttcaacaggggagagtgttga

SEQ ID NO: 74 - DNA, 336 bp, Artificial Sequence
  Synthethic Polynucleotide
gacgtagtactgacccaaagccccctttctctcccagtaaccctcggacaaccagcctcaatttcatgcagatcatcacaatcacttgagacgagcgacggagacacttttcttgagtggttccaacaaagacccggacaaagcccacgcctgcttatttacgaggtatcaagcagattctcaggagttccagacagattttcaggcagcggatccggcacagacttcacccttaaaattagcagagtagaagcagaagatgtaggagtgtattattgtatgcaagtcacccacgaccccctgaccttcggacaaggaactaagctcgaaatcaaa

SEQ ID NO: 75 - DNA, 660 bp, Artificial Sequence
  Synthethic Polynucleotide
gacgtagtactgacccaaagccccctttctctcccagtaaccctcggacaaccagcctcaatttcatgcagatcatcacaatcacttgagacgagcgacggagacacttttcttgagtggttccaacaaagacccggacaaagcccacgcctgcttatttacgaggtatcaagcagattctcaggagttccagacagattttcaggcagcggatccggcacagacttcacccttaaaattagcagagtagaagcagaagatgtaggagtgtattattgtatgcaagtcacccacgaccccctgaccttcggacaaggaactaagctcgaaatcaaaagaacggtggctgcaccatctgtcttcatcttcccgccatctgatgagcagttgaaatctggaactgcctctgttgtgtgcctgctgaataacttctatcccagagaggccaaagtacagtggaaggtggataacgccctccaatcgggtaactcccaggagagtgtcacagagcaggacagcaaggacagcacctacagcctcagcagcaccctgacgctgagcaaagcagactacgagaaacacaaagtctacgcctgcgaagtcacccatcagggcctgagctcgcccgtcacaaagagcttcaacaggggagagtgttga

SEQ ID NO: 76 - DNA, 336 bp, Artificial Sequence
  Synthethic Polynucleotide
gacgtagtactgacccaaagccccctttctctcccagtaaccctcggacaaccagcctcaatttcatgcagatcatcacaatcacttgagaccagcgacggagatacttttcttgagtggttccaacaaagacccggacaaagcccacgcctgcttatttacgaggtatcaaacagattctcaggagttccagacagattttcaggcagcggatccggcacagacttcacccttaaaattagcagagtagaagcagaagatgtaggagtgtattattgtttccaagtcacccacgaccccgtcacgttcggacaaggaactaagctcgaaatcaaa

SEQ ID NO: 77 - DNA, 660 bp, Artificial Sequence
  Synthethic Polynucleotide
gacgtagtactgacccaaagccccctttctctcccagtaaccctcggacaaccagcctcaatttcatgcagatcatcacaatcacttgagaccagcgacggagatacttttcttgagtggttccaacaaagacccggacaaagcccacgcctgcttatttacgaggtatcaaacagattctcaggagttccagacagattttcaggcagcggatccggcacagacttcacccttaaaattagcagagtagaagcagaagatgtaggagtgtattattgtttccaagtcacccacgaccccgtcacgttcggacaaggaactaagctcgaaatcaaaagaacggtggctgcaccatctgtcttcatcttcccgccatctgatgagcagttgaaatctggaactgcctctgttgtgtgcctgctgaataacttctatcccagagaggccaaagtacagtggaaggtggataacgccctccaatcgggtaactcccaggagagtgtcacagagcaggacagcaaggacagcacctacagcctcagcagcaccctgacgctgagcaaagcagactacgagaaacacaaagtctacgcctgcgaagtcacccatcagggcctgagctcgcccgtcacaaagagcttcaacaggggagagtgttga

SEQ ID NO: 78 - DNA, 336 bp, Artificial Sequence
  Synthethic Polynucleotide
gacgtagtactgacccaaagccccctttctctcccagtaaccctcggacaaccagcctcaatttcatgcagatcatcacaatcacttgagtccagcgacggagacacttttcttgagtggttccaacaaagacccggacaaagcccacgcctgcttatttacgatgtatcaactagattctcaggagttccagacagattttcaggcagcggatccggcacagacttcacccttaaaattagcagagtagaagcagaagatgtaggagtgtattattgttttcaagtcacccatgaccccgtgaccttcggacaaggaactaagctcgaaatcaaa

SEQ ID NO: 79 - DNA, 660 bp, Artificial Sequence
  Synthethic Polynucleotide
gacgtagtactgacccaaagccccctttctctcccagtaaccctcggacaaccagcctcaatttcatgcagatcatcacaatcacttgagtccagcgacggagacacttttcttgagtggttccaacaaagacccggacaaagcccacgcctgcttatttacgatgtatcaactagattctcaggagttccagacagattttcaggcagcggatccggcacagacttcacccttaaaattagcagagtagaagcagaagatgtaggagtgtattattgttttcaagtcacccatgaccccgtgaccttcggacaaggaactaagctcgaaatcaaaagaacggtggctgcaccatctgtcttcatcttcccgccatctgatgagcagttgaaatctggaactgcctctgttgtgtgcctgctgaataacttctatcccagagaggccaaagtacagtggaaggtggataacgccctccaatcgggtaactcccaggagagtgtcacagagcaggacagcaaggacagcacctacagcctcagcagcaccctgacgctgagcaaagcagactacgagaaacacaaagtctacgcctgcgaagtcacccatcagggcctgagctcgcccgtcacaaagagcttcaacaggggagagtgttga

SEQ ID NO: 80 - DNA, 336 bp, Artificial Sequence
  Synthethic Polynucleotide
gacgtagtactgacccaaagccccctttctctcccagtaaccctcggacaaccagcctcaatttcatgcagatcatcacaatcacttgaggaaagcgacggatacacttttcttgaatggttccaacaaagacccggacaaagcccacgcctgcttatttacgatgtatcagaaagattctcaggagttccagacagattttcaggcagcggatccggcacagacttcacccttaaaattagcagagtagaagcagaagatgtaggagtgtattattgtttccaagcgacctacgaccccctcaccttcggacaaggaactaagctcgaaatcaaa

SEQ ID NO: 81 - DNA, 660 bp, Artificial Sequence
  Synthethic Polynucleotide
gacgtagtactgacccaaagccccctttctctcccagtaaccctcggacaaccagcctcaatttcatgcagatcatcacaatcacttgaggaaagcgacggatacacttttcttgaatggttccaacaaagacccggacaaagcccacgcctgcttatttacgatgtatcagaaagattctcaggagttccagacagattttcaggcagcggatccggcacagacttcacccttaaaattagcagagtagaagcagaagatgtaggagtgtattattgtttccaagcgacctacgaccccctcaccttcggacaaggaactaagctcgaaatcaaaagaacggtggctgcaccatctgtcttcatcttcccgccatctgatgagcagttgaaatctggaactgcctctgttgtgtgcctgctgaataacttctatcccagagaggccaaagtacagtggaaggtggataacgccctccaatcgggtaactcccaggagagtgtcacagagcaggacagcaaggacagcacctacagcctcagcagcaccctgacgctgagcaaagcagactacgagaaacacaaagtctacgcctgcgaagtcacccatcagggcctgagctcgcccgtcacaaagagcttcaacaggggagagtgttga

SEQ ID NO: 82 - DNA, 345 bp, Artificial Sequence
  Synthethic Polynucleotide
gaagtacagttggtagaaagcggcggaggacttgtgcagccaggtggatctctcagactttcatgtgccgcaagcggttttacttttagttactatggaatgaactggattagacaagcgcccggaaaaggattggaatggataggcatgatatactacgacagctcggagaaacattatgccgactcagttaaaggaagatttacaatatcaagagacaatagcaaaaacacactttatcttcaaatgaattcactgcgagccgaggatacagcagtctattattgcgcaaaagggacgacgcccgattactggggtcaaggaacaatggtaaccgtgtcaagc

SEQ ID NO: 83 - DNA, 336 bp, Artificial Sequence
  Synthethic Polynucleotide
gacgtagtactgacccaaagccccctttctctcccagtaaccctcggacaaccagcctcaatttcatgcagatcatcacaatcacttgaggacagcgacggaggaacttttcttgagtggttccaacaaagacccggacaaagcccacgcctgcttatttacgacgtatcaagcagattctcaggagttccagacagattttcaggcagcggatccggcacagacttcacccttaaaattagcagagtagaagcagaagatgtaggagtgtattattgttttcaagcgacccacgaccccctgacgttcggacaaggaactaagctcgaaatcaaa

SEQ ID NO: 84 - DNA, 1338 bp, Artificial Sequence
  Synthethic Polynucleotide
gaagtacagttggtagaaagcggcggaggacttgtgcagccaggtggatctctcagactttcatgtgccgcaagcggttttacttttagttactatggaatgaactggattagacaagcgcccggaaaaggattggaatggataggcatgatatactacgacagctcggagaaacattatgccgactcagttaaaggaagatttacaatatcaagagacaatagcaaaaacacactttatcttcaaatgaattcactgcgagccgaggatacagcagtctattattgcgcaaaagggacgacgcccgattactggggtcaaggaacaatggtaaccgtgtcaagcgcgtcgaccaagggcccatcggtcttccccctggcaccctcctccaagagcacctctgggggcacagcggccctgggctgcctggtcaaggactacttccccgaaccggtgacggtgtcgtggaactcaggcgccctgaccagcggcgtgcacaccttcccggctgtcctacagtcctcaggactctactccctcagcagcgtggtgaccgtgccctccagcagcttgggcacccagacctacatctgcaacgtgaatcacaagcccagcaacaccaaggtggacaagaaagttgagcccaaatcttgtgacaaaactcacacatgcccaccgtgcccagcacctgaagccgcggggggaccgtcagtcttcctcttccccccaaaacccaaggacaccctcatgatctcccggacccctgaggtcacatgcgtggtggtggacgtgagccacgaagaccctgaggtcaagttcaactggtacgtggacggcgtggaggtgcataatgccaagacaaagccgcgggaggagcagtacaacagcacgtaccgtgtggtcagcgtcctcaccgtcctgcaccaggactggctgaatggcaaggagtacaagtgcaaggtctccaacaaagccctcccagcccccatcgagaaaaccatctccaaagccaaagggcagccccgagaaccacaggtgtacaccctgcccccatcccgcgaggagatgaccaagaaccaggtcagcctgacctgcctggtcaaaggcttctatcccagcgacatcgccgtggagtgggagagcaatgggcagccggagaacaactacaagaccacgcctcccgtgctggactccgacggctccttcttcctctacagcaagctcaccgtggacaagagcaggtggcagcaggggaacgtcttctcatgctccgtgatgcatgaggctctgcacaaccactacacgcagaagagcctctccctgtctccgggtaaatga

SEQ ID NO: 85 - DNA, 660 bp, Artificial Sequence
  Synthethic Polynucleotide
gacgtagtactgacccaaagccccctttctctcccagtaaccctcggacaaccagcctcaatttcatgcagatcatcacaatcacttgaggacagcgacggaggaacttttcttgagtggttccaacaaagacccggacaaagcccacgcctgcttatttacgacgtatcaagcagattctcaggagttccagacagattttcaggcagcggatccggcacagacttcacccttaaaattagcagagtagaagcagaagatgtaggagtgtattattgttttcaagcgacccacgaccccctgacgttcggacaaggaactaagctcgaaatcaaaagaacggtggctgcaccatctgtcttcatcttcccgccatctgatgagcagttgaaatctggaactgcctctgttgtgtgcctgctgaataacttctatcccagagaggccaaagtacagtggaaggtggataacgccctccaatcgggtaactcccaggagagtgtcacagagcaggacagcaaggacagcacctacagcctcagcagcaccctgacgctgagcaaagcagactacgagaaacacaaagtctacgcctgcgaagtcacccatcagggcctgagctcgcccgtcacaaagagcttcaacaggggagagtgttga

SEQ ID NO: 86 - DNA, 345 bp, Artificial Sequence
  Synthethic Polynucleotide
gaagtacagttggtagaaagcggcggaggacttgtgcagccaggtggatctctcagactttcatgtgccgcaagcggttttacttttagtaactatggaatgaactggataagacaagcgcccggaaaaggattggaatggataggcatgatatactacgacagctcggacaaacattatgccgactcagttaaaggaagatttacaatatcaagagacaatagcaaaaacacactttatcttcaaatgaattcactgcgagccgaggatacagcagtctattattgcgcaaaagggacgacgccggatgtatggggtcaaggaacaatggtaaccgtgtcaagc

SEQ ID NO: 87 - DNA, 336 bp, Artificial Sequence
  Synthethic Polynucleotide
gacgtagtactgacccaaagccccctttctctcccagtaaccctcggacaaccagcctcaatttcatgcagatcatcacaatcacttgaagagagcgacggatacacttttcttcattggttccaacaaagacccggacaaagcccacgcctgcttatttacgaggtatcaaacagattctcaggagttccagacagattttcaggcagcggatccggcacagacttcacccttaaaattagcagagtagaagcagaagatgtaggagtgtattattgtttccaagccacccacgaccccgtgacgttcggacaaggaactaagctcgaaatcaaa

SEQ ID NO: 88 - DNA, 1338 bp, Artificial Sequence
  Synthethic Polynucleotide
gaagtacagttggtagaaagcggcggaggacttgtgcagccaggtggatctctcagactttcatgtgccgcaagcggttttacttttagtaactatggaatgaactggataagacaagcgcccggaaaaggattggaatggataggcatgatatactacgacagctcggacaaacattatgccgactcagttaaaggaagatttacaatatcaagagacaatagcaaaaacacactttatcttcaaatgaattcactgcgagccgaggatacagcagtctattattgcgcaaaagggacgacgccggatgtatggggtcaaggaacaatggtaaccgtgtcaagcgcgtcgaccaagggcccatcggtcttccccctggcaccctcctccaagagcacctctgggggcacagcggccctgggctgcctggtcaaggactacttccccgaaccggtgacggtgtcgtggaactcaggcgccctgaccagcggcgtgcacaccttcccggctgtcctacagtcctcaggactctactccctcagcagcgtggtgaccgtgccctccagcagcttgggcacccagacctacatctgcaacgtgaatcacaagcccagcaacaccaaggtggacaagaaagttgagcccaaatcttgtgacaaaactcacacatgcccaccgtgcccagcacctgaagccgcggggggaccgtcagtcttcctcttccccccaaaacccaaggacaccctcatgatctcccggacccctgaggtcacatgcgtggtggtggacgtgagccacgaagaccctgaggtcaagttcaactggtacgtggacggcgtggaggtgcataatgccaagacaaagccgcgggaggagcagtacaacagcacgtaccgtgtggtcagcgtcctcaccgtcctgcaccaggactggctgaatggcaaggagtacaagtgcaaggtctccaacaaagccctcccagcccccatcgagaaaaccatctccaaagccaaagggcagccccgagaaccacaggtgtacaccctgcccccatcccgcgaggagatgaccaagaaccaggtcagcctgacctgcctggtcaaaggcttctatcccagcgacatcgccgtggagtgggagagcaatgggcagccggagaacaactacaagaccacgcctcccgtgctggactccgacggctccttcttcctctacagcaagctcaccgtggacaagagcaggtggcagcaggggaacgtcttctcatgctccgtgatgcatgaggctctgcacaaccactacacgcagaagagcctctccctgtctccgggtaaatga

SEQ ID NO: 89 - DNA, 660 bp, Artificial Sequence
  Synthethic Polynucleotide
gacgtagtactgacccaaagccccctttctctcccagtaaccctcggacaaccagcctcaatttcatgcagatcatcacaatcacttgaagagagcgacggatacacttttcttcattggttccaacaaagacccggacaaagcccacgcctgcttatttacgaggtatcaaacagattctcaggagttccagacagattttcaggcagcggatccggcacagacttcacccttaaaattagcagagtagaagcagaagatgtaggagtgtattattgtttccaagccacccacgaccccgtgacgttcggacaaggaactaagctcgaaatcaaaagaacggtggctgcaccatctgtcttcatcttcccgccatctgatgagcagttgaaatctggaactgcctctgttgtgtgcctgctgaataacttctatcccagagaggccaaagtacagtggaaggtggataacgccctccaatcgggtaactcccaggagagtgtcacagagcaggacagcaaggacagcacctacagcctcagcagcaccctgacgctgagcaaagcagactacgagaaacacaaagtctacgcctgcgaagtcacccatcagggcctgagctcgcccgtcacaaagagcttcaacaggggagagtgttga

SEQ ID NO: 90 - DNA, 345 bp, Artificial Sequence
  Synthethic Polynucleotide
gaagtacagttggtagaaagcggcggaggacttgtgcaaccaggtggatctctcagactttcatgtgccgcaagcggttttacttttagtaactatggaatgaactgggttagacaagcgcccggaaaaggattggaatggataggcatgatatattacgacagctcggagaaacattatgccgactcagttaaaggaagatttacaatatcaagagacaatagcaaaaacacactttatcttcaaatgaattcactgcgagccgaggatacagcagtctattattgcgcaaaagggaccacccccgattactggggtcaaggaacaatggtaaccgtgtcaagc

SEQ ID NO: 91 - DNA, 336 bp, Artificial Sequence
  Synthethic Polynucleotide
gacgtagtactgacccaaagccccctttctctcccagtaaccctcggacaaccagcctcaatttcatgcagatcatcacaatcacttgaagaaagcgacggatacacttttcttcactggttccaacaaagacccggacaaagcccacgcctgcttatttacgaggtatcaaccagattctcaggagttccagacagattttcaggcagcggatccggcacagacttcacccttaaaattagcagagtagaagcagaagatgtaggagtgtattattgtttccaagccacccacgaccccctgaccttcggacaaggaactaagctcgaaatcaaa

SEQ ID NO: 92 - DNA, 1338 bp, Artificial Sequence
  Synthethic Polynucleotide
gaagtacagttggtagaaagcggcggaggacttgtgcaaccaggtggatctctcagactttcatgtgccgcaagcggttttacttttagtaactatggaatgaactgggttagacaagcgcccggaaaaggattggaatggataggcatgatatattacgacagctcggagaaacattatgccgactcagttaaaggaagatttacaatatcaagagacaatagcaaaaacacactttatcttcaaatgaattcactgcgagccgaggatacagcagtctattattgcgcaaaagggaccacccccgattactggggtcaaggaacaatggtaaccgtgtcaagcgcgtcgaccaagggcccatcggtcttccccctggcaccctcctccaagagcacctctgggggcacagcggccctgggctgcctggtcaaggactacttccccgaaccggtgacggtgtcgtggaactcaggcgccctgaccagcggcgtgcacaccttcccggctgtcctacagtcctcaggactctactccctcagcagcgtggtgaccgtgccctccagcagcttgggcacccagacctacatctgcaacgtgaatcacaagcccagcaacaccaaggtggacaagaaagttgagcccaaatcttgtgacaaaactcacacatgcccaccgtgcccagcacctgaagccgcggggggaccgtcagtcttcctcttccccccaaaacccaaggacaccctcatgatctcccggacccctgaggtcacatgcgtggtggtggacgtgagccacgaagaccctgaggtcaagttcaactggtacgtggacggcgtggaggtgcataatgccaagacaaagccgcgggaggagcagtacaacagcacgtaccgtgtggtcagcgtcctcaccgtcctgcaccaggactggctgaatggcaaggagtacaagtgcaaggtctccaacaaagccctcccagcccccatcgagaaaaccatctccaaagccaaagggcagccccgagaaccacaggtgtacaccctgcccccatcccgcgaggagatgaccaagaaccaggtcagcctgacctgcctggtcaaaggcttctatcccagcgacatcgccgtggagtgggagagcaatgggcagccggagaacaactacaagaccacgcctcccgtgctggactccgacggctccttcttcctctacagcaagctcaccgtggacaagagcaggtggcagcaggggaacgtcttctcatgctccgtgatgcatgaggctctgcacaaccactacacgcagaagagcctctccctgtctccgggtaaatga

SEQ ID NO: 93 - DNA, 660 bp, Artificial Sequence
  Synthethic Polynucleotide
gacgtagtactgacccaaagccccctttctctcccagtaaccctcggacaaccagcctcaatttcatgcagatcatcacaatcacttgaagaaagcgacggatacacttttcttcactggttccaacaaagacccggacaaagcccacgcctgcttatttacgaggtatcaaccagattctcaggagttccagacagattttcaggcagcggatccggcacagacttcacccttaaaattagcagagtagaagcagaagatgtaggagtgtattattgtttccaagccacccacgaccccctgaccttcggacaaggaactaagctcgaaatcaaaagaacggtggctgcaccatctgtcttcatcttcccgccatctgatgagcagttgaaatctggaactgcctctgttgtgtgcctgctgaataacttctatcccagagaggccaaagtacagtggaaggtggataacgccctccaatcgggtaactcccaggagagtgtcacagagcaggacagcaaggacagcacctacagcctcagcagcaccctgacgctgagcaaagcagactacgagaaacacaaagtctacgcctgcgaagtcacccatcagggcctgagctcgcccgtcacaaagagcttcaacaggggagagtgttga

SEQ ID NO: 94 - DNA, 1338 bp, Artificial Sequence
  Synthethic Polynucleotide
gaagtacagttggtagaaagcggcggaggacttgtgcaaccaggtggatctctcagactttcatgtgccgcaagcggttttacttttagtaactatggaatgaactgggttagacaagcgcccggaaaaggattggaatggataggcatgatatattacgacagctcggagaaacattatgccgactcagttaaaggaagatttacaatatcaagagacaatagcaaaaacacactttatcttcaaatgaattcactgcgagccgaggatacagcagtctattattgcgcaaaagggaccacccccgattactggggtcaaggaacaatggtaaccgtgtcaagcgcgtcgaccaagggcccatcggtcttccccctggcaccctcctccaagagcacctctgggggcacagcggccctgggctgcctggtcaaggactacttccccgaaccggtgacggtgtcgtggaactcaggcgccctgaccagcggcgtgcacaccttcccggctgtcctacagtcctcaggactctactccctcagcagcgtggtgaccgtgccctccagcagcttgggcacccagacctacatctgcaacgtgaatcacaagcccagcaacaccaaggtggacaagaaagttgagcccaaatcttgtgacaaaactcacacatgcccaccgtgcccagcacctgaagccgcggggggaccgtcagtcttcctcttccccccaaaacccaaggaccaactcatgatctcccggacccctgaggtcacatgcgtggtggtggacgtgagccacgaagaccctgaggtcaagttcaactggtacgtggacggcgtggaggtgcataatgccaagacaaagccgcgggaggagcagtacaacagcacgtaccgtgtggtcagcgtcctcaccgtcctgcaccaggactggctgaatggcaaggagtacaagtgcaaggtctccaacaaagccctcccagcccccatcgagaaaaccatctccaaagccaaagggcagccccgagaaccacaggtgtacaccctgcccccatcccgcgaggagatgaccaagaaccaggtcagcctgacctgcctggtcaaaggcttctatcccagcgacatcgccgtggagtgggagagcaatgggcagccggagaacaactacaagaccacgcctcccgtgctggactccgacggctccttcttcctctacagcaagctcaccgtggacaagagcaggtggcagcaggggaacgtcttctcatgctccgtgctgcatgaggctctgcacaaccactacacgcagaagagcctctccctgtctccgggtaaatga

SEQ ID NO: 95 - DNA, 336 bp, Artificial Sequence
  Synthethic Polynucleotide
gacgtagtactgacccaaagccccctttctctcccagtaaccctcggacaaccagcctcaatttcatgcagatcatcacaatcacttgcggacagcgacggagatacttttcttcactggttccaacaaagacccggacaaagcccacgcctgcttatttacgcggtatcacacagattctcaggagttccagacagattttcaggcagcggatccggcacagacttcacccttaaaattagcagagtagaagcagaagatgtaggagtgtattattgtttccaagccacccatgaccccgtcacgttcggacaaggaactaagctcgaaatcaaa

SEQ ID NO: 96 - DNA, 660 bp, Artificial Sequence
  Synthethic Polynucleotide
gacgtagtactgacccaaagccccctttctctcccagtaaccctcggacaaccagcctcaatttcatgcagatcatcacaatcacttgcggacagcgacggagatacttttcttcactggttccaacaaagacccggacaaagcccacgcctgcttatttacgcggtatcacacagattctcaggagttccagacagattttcaggcagcggatccggcacagacttcacccttaaaattagcagagtagaagcagaagatgtaggagtgtattattgtttccaagccacccatgaccccgtcacgttcggacaaggaactaagctcgaaatcaaaagaacggtggctgcaccatctgtcttcatcttcccgccatctgatgagcagttgaaatctggaactgcctctgttgtgtgcctgctgaataacttctatcccagagaggccaaagtacagtggaaggtggataacgccctccaatcgggtaactcccaggagagtgtcacagagcaggacagcaaggacagcacctacagcctcagcagcaccctgacgctgagcaaagcagactacgagaaacacaaagtctacgcctgcgaagtcacccatcagggcctgagctcgcccgtcacaaagagcttcaacaggggagagtgttga

SEQ ID NO: 97 - DNA, 345 bp, Artificial Sequence
  Synthethic Polynucleotide
gaagtacagttggtagaaagcggcggaggacttgtgcagccaggtggatctctcagactttcatgtgccgcaagcggttttacttttagtaactatggaatgaactgggttagacaagcgcccggaaaaggattggaatggataggcatgatatactacgacagctccgagaaacattatgccgactcagttaaaggaagatttacaatatcaagagacaatagcaaaaacacactttatcttcaaatgaattcactgcgagccgaggatacagcagtctattattgcgcaaaaggcacgacgcccgataaatggggtcaaggaacaatggtaaccgtgtcaagc

SEQ ID NO: 98 - DNA, 336 bp, Artificial Sequence
  Synthethic Polynucleotide
gacgtagtactgacccaaagccccctttctctcccagtaaccctcggacaaccagcctcaatttcatgcagatcatcacaatcacttgaggagagcgacggatacacttttcttgagtggttccaacaaagacccggacaaagcccacgcctgcttatttacgaggtatcacatagattctcaggagttccagacagattttcaggcagcggatccggcacagacttcacccttaaaattagcagagtagaagcagaagatgtaggagtgtattattgtttccaagcgacccacgaccccctgacgttcggacaaggaactaagctcgaaatcaaa

SEQ ID NO: 99 - DNA, 1338 bp, Artificial Sequence
  Synthethic Polynucleotide
gaagtacagttggtagaaagcggcggaggacttgtgcagccaggtggatctctcagactttcatgtgccgcaagcggttttacttttagtaactatggaatgaactgggttagacaagcgcccggaaaaggattggaatggataggcatgatatactacgacagctccgagaaacattatgccgactcagttaaaggaagatttacaatatcaagagacaatagcaaaaacacactttatcttcaaatgaattcactgcgagccgaggatacagcagtctattattgcgcaaaaggcacgacgcccgataaatggggtcaaggaacaatggtaaccgtgtcaagcgcgtcgaccaagggcccatcggtcttccccctggcaccctcctccaagagcacctctgggggcacagcggccctgggctgcctggtcaaggactacttccccgaaccggtgacggtgtcgtggaactcaggcgccctgaccagcggcgtgcacaccttcccggctgtcctacagtcctcaggactctactccctcagcagcgtggtgaccgtgccctccagcagcttgggcacccagacctacatctgcaacgtgaatcacaagcccagcaacaccaaggtggacaagaaagttgagcccaaatcttgtgacaaaactcacacatgcccaccgtgcccagcacctgaagccgcggggggaccgtcagtcttcctcttccccccaaaacccaaggacaccctcatgatctcccggacccctgaggtcacatgcgtggtggtggacgtgagccacgaagaccctgaggtcaagttcaactggtacgtggacggcgtggaggtgcataatgccaagacaaagccgcgggaggagcagtacaacagcacgtaccgtgtggtcagcgtcctcaccgtcctgcaccaggactggctgaatggcaaggagtacaagtgcaaggtctccaacaaagccctcccagcccccatcgagaaaaccatctccaaagccaaagggcagccccgagaaccacaggtgtacaccctgcccccatcccgcgaggagatgaccaagaaccaggtcagcctgacctgcctggtcaaaggcttctatcccagcgacatcgccgtggagtgggagagcaatgggcagccggagaacaactacaagaccacgcctcccgtgctggactccgacggctccttcttcctctacagcaagctcaccgtggacaagagcaggtggcagcaggggaacgtcttctcatgctccgtgatgcatgaggctctgcacaaccactacacgcagaagagcctctccctgtctccgggtaaatga

SEQ ID NO: 100 - DNA, 660 bp, Artificial Sequence
  Synthethic Polynucleotide
gacgtagtactgacccaaagccccctttctctcccagtaaccctcggacaaccagcctcaatttcatgcagatcatcacaatcacttgaggagagcgacggatacacttttcttgagtggttccaacaaagacccggacaaagcccacgcctgcttatttacgaggtatcacatagattctcaggagttccagacagattttcaggcagcggatccggcacagacttcacccttaaaattagcagagtagaagcagaagatgtaggagtgtattattgtttccaagcgacccacgaccccctgacgttcggacaaggaactaagctcgaaatcaaaagaacggtggctgcaccatctgtcttcatcttcccgccatctgatgagcagttgaaatctggaactgcctctgttgtgtgcctgctgaataacttctatcccagagaggccaaagtacagtggaaggtggataacgccctccaatcgggtaactcccaggagagtgtcacagagcaggacagcaaggacagcacctacagcctcagcagcaccctgacgctgagcaaagcagactacgagaaacacaaagtctacgcctgcgaagtcacccatcagggcctgagctcgcccgtcacaaagagcttcaacaggggagagtgttga

SEQ ID NO: 101 - DNA, 345 bp, Artificial Sequence
  Synthethic Polynucleotide
gaagtacagttggtagaaagcggcggaggacttgtgcagccaggtggatctctcagactttcatgtgccgcaagcggttttacttttagtaactatggaatgaactgggttagacaagcgcccggaaaaggattggaatggataggaatgatatactacgacagctccgagaaacattatgccgactcagttaaaggaagatttacaatatcaagagacaatagcaaaaacacactttatcttcaaatgaattcactgcgagccgaggatacagcagtctattattgcgcaaaaggctcgacccccgattactggggtcaaggaacaatggtaaccgtgtcaagc

SEQ ID NO: 102 - DNA, 336 bp, Artificial Sequence
  Synthethic Polynucleotide
gacgtagtactgacccaaagccccctttctctcccagtaaccctcggacaaccagcctcaatttcatgcagatcatcacaatcacttgaggacagcgacggaggcacttttcttgagtggttccaacaaagacccggacaaagcccacgcctgcttatttacgacgtatcaagcagattctcaggagttccagacagattttcaggcagcggatccggcacagacttcacccttaaaattagcagagtagaagcagaagatgtaggagtgtattattgtttccaagccacccacgaccccctcagcttcggacaaggaactaagctcgaaatcaaa

SEQ ID NO: 103 - protein, 330 aa, Homo sapiens [sequence omitted]

SEQ ID NO: 104 - protein, 19 aa, Artificial Sequence
  Synthethic Polypeptide
MEFGLSWLFLVAILKGVQC

SEQ ID NO: 105 - protein, 5 aa, Artificial Sequence
  Synthethic Polypeptide
  misc_feature (1)..(1): Xaa can be Asn or Tyr
XYGMN

SEQ ID NO: 106 - protein, 17 aa, Artificial Sequence
  Synthethic Polypeptide
  misc_feature (8)..(8): Xaa can be Glu or Asp
MIYYDSSXKHYADSVKG

SEQ ID NO: 107 - protein, 6 aa, Artificial Sequence
  Synthethic Polypeptide
  misc_feature (2)..(2): Xaa can be Thr or Ser
  misc_feature (6)..(6): Xaa can be Tyr, Val, or Lys
GXTPDX

SEQ ID NO: 108 - protein, 16 aa, Artificial Sequence
  Synthethic Polypeptide
  misc_feature (7)..(7): Xaa can be Ala or Glu
  misc_feature (8)..(8): Xaa can be Thr, Ser, Glu, or Asp
  misc_feature (12)..(12): Xaa can be Asp, Tyr, or Gly
  misc_feature (16)..(16): Xaa can be Glu or His
RSSQSLXXSDGXTFLX

SEQ ID NO: 109 - protein, 7 aa, Artificial Sequence
  Synthethic Polypeptide
  misc_feature (1)..(1): Xaa can be Glu, Asp, or Ala
  misc_feature (4)..(4): Xaa can Asn, Ser, Thr, Glu, or His
XVSXRFS

SEQ ID NO: 110 - protein, 9 aa, Artificial Sequence
  Synthethic Polypeptide
  misc_feature (1)..(1): Xaa can be Phe or Met
  misc_feature (3)..(3): Xaa can be Val or Ala
  misc_feature (5)..(5): Xaa can be His or Tyr
  misc_feature (8)..(8): Xaa can be Met, Leu, or Val
  misc_feature (9)..(9): Xaa can be Thr or Ser
XQXTXDPXX

SEQ ID NO: 111 - protein, 329 aa, Artificial Sequence
  Synthetic Polypeptide
ASTKGPSVFPLAPSSKSTSGGTAALGCLVKDYFPEPVTVSWNSGALTSGVHTFPAVLQSSGLYSLSSVVTVPSSSLGTQTYICNVNHKPSNTKVDKKVEPKSCDKTHTCPPCPAPELLGGPSVFLFPPKPKDTLMISRTPEVTCVVVDVSHEDPEVKFNWYVDGVEVHNAKTKPREEQYNSTYRVVSVLTVLHQDWLNGKEYKCKVSNKALPAPIEKTISKAKGQPREPQVYTLPPSRDELTKNQVSLTCLVKGFYPSDIAVEWESNGQPENNYKTTPPVLDSDGSFFLYSKLTVDKSRWQQGNVFSCSVMHEALHNHYTQKSLSLSPG

SEQ ID NO: 112 - protein, 329 aa, Artificial Sequence
  Synthetic Polypeptide
ASTKGPSVFPLAPSSKSTSGGTAALGCLVKDYFPEPVTVSWNSGALTSGVHTFPAVLQSSGLYSLSSVVTVPSSSLGTQTYICNVNHKPSNTKVDKKVEPKSCDKTHTCPPCPAPEAAGGPSVFLFPPKPKDTLMISRTPEVTCVVVDVSHEDPEVKFNWYVDGVEVHNAKTKPREEQYNSTYRVVSVLTVLHQDWLNGKEYKCKVSNKALPAPIEKTISKAKGQPREPQVYTLPPSRDELTKNQVSLTCLVKGFYPSDIAVEWESNGQPENNYKTTPPVLDSDGSFFLYSKLTVDKSRWQQGNVFSCSVMHEALHNHYTQKSLSLSPG

SEQ ID NO: 113 - protein, 329 aa, Artificial Sequence
  Synthetic Polypeptide
ASTKGPSVFPLAPSSKSTSGGTAALGCLVKDYFPEPVTVSWNSGALTSGVHTFPAVLQSSGLYSLSSVVTVPSSSLGTQTYICNVNHKPSNTKVDKKVEPKSCDKTHTCPPCPAPEAAGGPSVFLFPPKPKDQLMISRTPEVTCVVVDVSHEDPEVKFNWYVDGVEVHNAKTKPREEQYNSTYRVVSVLTVLHQDWLNGKEYKCKVSNKALPAPIEKTISKAKGQPREPQVYTLPPSREEMTKNQVSLTCLVKGFYPSDIAVEWESNGQPENNYKTTPPVLDSDGSFFLYSKLTVDKSRWQQGNVFSCSVLHEALHNHYTQKSLSLSPG

SEQ ID NO: 114 - protein, 444 aa, Artificial Sequence
  Synthetic Polypeptide
EVQLVESGGGLVQPGGSLRLSCAASGFTFSNYGMNWIRQAPGKGLEWIGMIYYDSSEKHYADSVKGRFTISRDNSKNTLYLQMNSLRAEDTAVYYCAKGTTPDYWGQGTMVTVSSASTKGPSVFPLAPSSKSTSGGTAALGCLVKDYFPEPVTVSWNSGALTSGVHTFPAVLQSSGLYSLSSVVTVPSSSLGTQTYICNVNHKPSNTKVDKKVEPKSCDKTHTCPPCPAPEAAGGPSVFLFPPKPKDTLMISRTPEVTCVVVDVSHEDPEVKFNWYVDGVEVHNAKTKPREEQYNSTYRVVSVLTVLHQDWLNGKEYKCKVSNKALPAPIEKTISKAKGQPREPQVYTLPPSREEMTKNQVSLTCLVKGFYPSDIAVEWESNGQPENNYKTTPPVLDSDGSFFLYSKLTVDKSRWQQGNVFSCSVMHEALHNHYTQKSLSLSPG

SEQ ID NO: 115 - protein, 444 aa, Artificial Sequence
  Synthetic Polypeptide
EVQLVESGGGLVQPGGSLRLSCAASGFTFSYYGMNWIRQAPGKGLEWIGMIYYDSSEKHYADSVKGRFTISRDNSKNTLYLQMNSLRAEDTAVYYCAKGTTPDYWGQGTMVTVSSASTKGPSVFPLAPSSKSTSGGTAALGCLVKDYFPEPVTVSWNSGALTSGVHTFPAVLQSSGLYSLSSVVTVPSSSLGTQTYICNVNHKPSNTKVDKKVEPKSCDKTHTCPPCPAPEAAGGPSVFLFPPKPKDTLMISRTPEVTCVVVDVSHEDPEVKFNWYVDGVEVHNAKTKPREEQYNSTYRVVSVLTVLHQDWLNGKEYKCKVSNKALPAPIEKTISKAKGQPREPQVYTLPPSREEMTKNQVSLTCLVKGFYPSDIAVEWESNGQPENNYKTTPPVLDSDGSFFLYSKLTVDKSRWQQGNVFSCSVMHEALHNHYTQKSLSLSPG

SEQ ID NO: 116 - protein, 444 aa, Artificial Sequence
  Synthetic Polypeptide
EVQLVESGGGLVQPGGSLRLSCAASGFTFSNYGMNWIRQAPGKGLEWIGMIYYDSSDKHYADSVKGRFTISRDNSKNTLYLQMNSLRAEDTAVYYCAKGTTPDVWGQGTMVTVSSASTKGPSVFPLAPSSKSTSGGTAALGCLVKDYFPEPVTVSWNSGALTSGVHTFPAVLQSSGLYSLSSVVTVPSSSLGTQTYICNVNHKPSNTKVDKKVEPKSCDKTHTCPPCPAPEAAGGPSVFLFPPKPKDTLMISRTPEVTCVVVDVSHEDPEVKFNWYVDGVEVHNAKTKPREEQYNSTYRVVSVLTVLHQDWLNGKEYKCKVSNKALPAPIEKTISKAKGQPREPQVYTLPPSREEMTKNQVSLTCLVKGFYPSDIAVEWESNGQPENNYKTTPPVLDSDGSFFLYSKLTVDKSRWQQGNVFSCSVMHEALHNHYTQKSLSLSPG

SEQ ID NO: 117 - protein, 444 aa, Artificial Sequence
  Synthetic Polypeptide
EVQLVESGGGLVQPGGSLRLSCAASGFTFSNYGMNWVRQAPGKGLEWIGMIYYDSSEKHYADSVKGRFTISRDNSKNTLYLQMNSLRAEDTAVYYCAKGTTPDYWGQGTMVTVSSASTKGPSVFPLAPSSKSTSGGTAALGCLVKDYFPEPVTVSWNSGALTSGVHTFPAVLQSSGLYSLSSVVTVPSSSLGTQTYICNVNHKPSNTKVDKKVEPKSCDKTHTCPPCPAPEAAGGPSVFLFPPKPKDTLMISRTPEVTCVVVDVSHEDPEVKFNWYVDGVEVHNAKTKPREEQYNSTYRVVSVLTVLHQDWLNGKEYKCKVSNKALPAPIEKTISKAKGQPREPQVYTLPPSREEMTKNQVSLTCLVKGFYPSDIAVEWESNGQPENNYKTTPPVLDSDGSFFLYSKLTVDKSRWQQGNVFSCSVMHEALHNHYTQKSLSLSPG

SEQ ID NO: 118 - protein, 444 aa, Artificial Sequence
  Synthetic Polypeptide
EVQLVESGGGLVQPGGSLRLSCAASGFTFSNYGMNWVRQAPGKGLEWIGMIYYDSSEKHYADSVKGRFTISRDNSKNTLYLQMNSLRAEDTAVYYCAKGTTPDYWGQGTMVTVSSASTKGPSVFPLAPSSKSTSGGTAALGCLVKDYFPEPVTVSWNSGALTSGVHTFPAVLQSSGLYSLSSVVTVPSSSLGTQTYICNVNHKPSNTKVDKKVEPKSCDKTHTCPPCPAPEAAGGPSVFLFPPKPKDQLMISRTPEVTCVVVDVSHEDPEVKFNWYVDGVEVHNAKTKPREEQYNSTYRVVSVLTVLHQDWLNGKEYKCKVSNKALPAPIEKTISKAKGQPREPQVYTLPPSREEMTKNQVSLTCLVKGFYPSDIAVEWESNGQPENNYKTTPPVLDSDGSFFLYSKLTVDKSRWQQGNVFSCSVLHEALHNHYTQKSLSLSPG

SEQ ID NO: 119 - protein, 444 aa, Artificial Sequence
  Synthetic Polypeptide
EVQLVESGGGLVQPGGSLRLSCAASGFTFSNYGMNWVRQAPGKGLEWIGMIYYDSSEKHYADSVKGRFTISRDNSKNTLYLQMNSLRAEDTAVYYCAKGTTPDKWGQGTMVTVSSASTKGPSVFPLAPSSKSTSGGTAALGCLVKDYFPEPVTVSWNSGALTSGVHTFPAVLQSSGLYSLSSVVTVPSSSLGTQTYICNVNHKPSNTKVDKKVEPKSCDKTHTCPPCPAPEAAGGPSVFLFPPKPKDTLMISRTPEVTCVVVDVSHEDPEVKFNWYVDGVEVHNAKTKPREEQYNSTYRVVSVLTVLHQDWLNGKEYKCKVSNKALPAPIEKTISKAKGQPREPQVYTLPPSREEMTKNQVSLTCLVKGFYPSDIAVEWESNGQPENNYKTTPPVLDSDGSFFLYSKLTVDKSRWQQGNVFSCSVMHEALHNHYTQKSLSLSPG

SEQ ID NO: 120 - protein, 444 aa, Artificial Sequence
  Synthetic Polypeptide
EVQLVESGGGLVQPGGSLRLSCAASGFTFSNYGMNWVRQAPGKGLEWIGMIYYDSSEKHYADSVKGRFTISRDNSKNTLYLQMNSLRAEDTAVYYCAKGSTPDYWGQGTMVTVSSASTKGPSVFPLAPSSKSTSGGTAALGCLVKDYFPEPVTVSWNSGALTSGVHTFPAVLQSSGLYSLSSVVTVPSSSLGTQTYICNVNHKPSNTKVDKKVEPKSCDKTHTCPPCPAPEAAGGPSVFLFPPKPKDTLMISRTPEVTCVVVDVSHEDPEVKFNWYVDGVEVHNAKTKPREEQYNSTYRVVSVLTVLHQDWLNGKEYKCKVSNKALPAPIEKTISKAKGQPREPQVYTLPPSREEMTKNQVSLTCLVKGFYPSDIAVEWESNGQPENNYKTTPPVLDSDGSFFLYSKLTVDKSRWQQGNVFSCSVMHEALHNHYTQKSLSLSPG

SEQ ID NO: 121 - protein, 14 aa, Artificial Sequence
  Synthetic
SSPMALGANATATR

SEQ ID NO: 122 - protein, 14 aa, Artificial Sequence
  Synthetic
TSSPMALGANATAT

SEQ ID NO: 123 - protein, 364 aa, Artificial Sequence
  Synthetic
QCKILRCNAEYVSSTLSLRGGGSSGALRGGGGGGRGGGVGSGGLCRALRSYALCTRRTARTCRGDLAFHSAVHGIEDLMIQHNCSRQGPTPPPPRGPALPGAGSGLPAPDPCDYEGRFSRLHGRPPGFLHCASFGDPHVRSFHHHFHTCRVQGAWPLLDNDFLFVQATSSPMALGANATATRKLTIIFKNMQECIDQKVYQAEVDNLPVAFEDGSINGGDRPGGSSLSIQTANPGNHVEIQAAYIGTTIIIRQTAGQLSFSIKVAEDVAMAFSAEQDLQLCVGGCPPSQRLSRSERNRRGAITIDTARRLCKEGLPVEDAYFHSCVFDVLISGDPNFTVAAQAALEDARAFLPDLEKLHLFPSD

SEQ ID NO: 124 - protein, 21 aa, Artificial Sequence
  Synthetic
SSPMALGANATATRKLTIIFK

SEQ ID NO: 125 - protein, 30 aa, Artificial Sequence
  Synthetic
DNDFLFVQATSSPMALGANATTRKLTIIFK

SEQ ID NO: 126 - protein, 21 aa, Artificial Sequence
  Synthetic
QLCVGGCPPSQRLSRSERNRR

SEQ ID NO: 127 - protein, 12 aa, Artificial Sequence
  Synthetic
SQRLSRSERNRR

SEQ ID NO: 128 - protein, 426 aa, Homo sapiens
MGEPGQSPSPRSSHGSPPTLSTLTLLLLLCGHAHSQCKILRCNAEYVSSTLSLRGGGSSGALRGGGGGGRGGGVGSGGLCRALRSYALCTRRTARTCRGDLAFHSAVHGIEDLMIQHNCSRQGPTAPPPPRGPALPGAGSGLPAPDPCDYEGRFSRLHGRPPGFLHCASFGDPHVRSFHHHFHTCRVQGAWPLLDNDFLFVQATSSPMALGANATATRKLTIIFKNMQECIDQKVYQAEVDNLPVAFEDGSINGGDRPGGSSLSIQTANPGNHVEIQAAYIGTTIIIRQTAGQLSFSIKVAEDVAMAFSAEQDLQLCVGGCPPSQRLSRSERNRRGAITIDTARRLCKEGLPVEDAYFHSCVFDVLISGDPNFTVAAQAALEDARAFLPDLEKLHLFPSDAGVPLSSATLLAPLLSGLFVLWLCIQ

SEQ ID NO: 129 - protein, 25 aa, Artificial Sequence
  Synthetic
DTHFPICIFCCGCCHRSKCGMCCKT